European Patent Specification EP 4 045 478 B1, published January 28, 2026. Title: CURCUMINOID COMPOSITION AND ITS THERAPEUTIC POTENTIAL  IN MANAGING LUNG FIBROSIS. Applicant: Majeed, Muhammed Nagabhushanam, Kalyanam Mundkur, Lakshmi Ramanujam, Rajendran. The sequence listing filed with the application follows.

SEQUENCE LISTING (8 sequences)

SEQ ID NO: 1 - DNA, 21 bp, Artificial Sequence
  Forward Primer of m Cola1
ttccctggacctaagggtact

SEQ ID NO: 2 - DNA, 18 bp, Artificial Sequence
  Reverse Primer of m Cola1
ttgagctccagcttcgcc

SEQ ID NO: 3 - DNA, 20 bp, Artificial Sequence
  Forward Primer for IL6
ggccttccctacttcacaag

SEQ ID NO: 4 - DNA, 20 bp, Artificial Sequence
  Reverse primer for IL6
atttccacgatttcccagag

SEQ ID NO: 5 - DNA, 24 bp, Artificial Sequence
  Forward Primer for IFN-gamma
tgaacgctacacactgcatcttgg

SEQ ID NO: 6 - DNA, 23 bp, Artificial Sequence
  Reverse Primer for IFN-gamma
cgactccttttccgcttcctgag

SEQ ID NO: 7 - DNA, 21 bp, Artificial Sequence
  Forward Primer for 18s rRNA
cgccgctagaggtgaaattct

SEQ ID NO: 8 - DNA, 21 bp, Artificial Sequence
  Reverse Primer for 18s rRNA
cgaacctccgactttcgttct